European Patent Specification EP 3 514 169 B1, published March 6, 2024. Title: Designed repeat proteins binding to serum albumin. Applicant: Molecular Partners AG. The sequence listing filed with the application follows.

SEQUENCE LISTING (54 sequences)

SEQ ID NO: 1 - protein, 32 aa, Artificial Sequence
  Synthetic Construct
GSDLGKKLLEAARAGQDDEVRILMANGADVNA

SEQ ID NO: 2 - protein, 28 aa, Artificial Sequence
  Synthetic Construct
QDKFGKTAFDISIDNGNEDLAEILQKLN

SEQ ID NO: 3 - protein, 28 aa, Artificial Sequence
  Synthetic Construct
QDKFGKTPFDLAIREGHEDIAEVLQKAA

SEQ ID NO: 4 - protein, 28 aa, Artificial Sequence
  Synthetic Construct
QDKFGKTPFDLAIDNGNEDIAEVLQKAA

SEQ ID NO: 5 - protein, 30 aa, Artificial Sequence
  Synthetic Construct
  misc_feature (1)..(1): Xaa can be any naturally occurring amino acid
  misc_feature (3)..(3): Xaa can be any naturally occurring amino acid
  misc_feature (22)..(22): Xaa can be any naturally occurring amino acid
  misc_feature (24)..(24): Xaa can be any naturally occurring amino acid
XLXKKLLEAARAGQDDEVRILXAXGADVNA

SEQ ID NO: 6 - protein, 28 aa, Artificial Sequence
  Synthetic Construct
  misc_feature (1)..(1): Xaa can be any naturally occurring amino acid
  misc_feature (4)..(4): Xaa can be any naturally occurring amino acid
  misc_feature (8)..(9): Xaa can be any naturally occurring amino acid
  misc_feature (11)..(13): Xaa can be any naturally occurring amino acid
  misc_feature (15)..(15): Xaa can be any naturally occurring amino acid
  misc_feature (17)..(17): Xaa can be any naturally occurring amino acid
  misc_feature (20)..(20): Xaa can be any naturally occurring amino acid
  misc_feature (23)..(23): Xaa can be any naturally occurring amino acid
XDKXGKTXXDXXXDXGXEDXAEXLQKAA

SEQ ID NO: 7 - protein, 28 aa, Artificial Sequence
  Synthetic Construct
  misc_feature (1)..(1): Xaa can be any naturally occurring amino acid
  misc_feature (4)..(4): Xaa can be any naturally occurring amino acid
  misc_feature (8)..(8): Xaa can be any naturally occurring amino acid
  misc_feature (11)..(13): Xaa can be any naturally occurring amino acid
  misc_feature (15)..(15): Xaa can be any naturally occurring amino acid
  misc_feature (17)..(17): Xaa can be any naturally occurring amino acid
  misc_feature (20)..(20): Xaa can be any naturally occurring amino acid
  misc_feature (23)..(23): Xaa can be any naturally occurring amino acid
XDKXGKTXADXXXDXGXEDXAEXLQKAA

SEQ ID NO: 8 - protein, 28 aa, Artificial Sequence
  Synthetic Construct
  misc_feature (1)..(1): Xaa can be any naturally occurring amino acid
  misc_feature (4)..(4): Xaa can be any naturally occurring amino acid
  misc_feature (8)..(8): Xaa can be any naturally occurring amino acid
  misc_feature (11)..(12): Xaa can be any naturally occurring amino acid
  misc_feature (15)..(15): Xaa can be any naturally occurring amino acid
  misc_feature (17)..(17): Xaa can be any naturally occurring amino acid
  misc_feature (20)..(20): Xaa can be any naturally occurring amino acid
  misc_feature (23)..(23): Xaa can be any naturally occurring amino acid
XDKXGKTXADXXADXGXEDXAEXLQKAA

SEQ ID NO: 9 - protein, 28 aa, Artificial Sequence
  Synthetic Construct
QDKSGKTPADLAADAGHEDIAEVLQKAA

SEQ ID NO: 10 - protein, 33 aa, Artificial Sequence
  Synthetic Construct
  misc_feature (1)..(1): Xaa can be any naturally occurring amino acid
  misc_feature (3)..(4): Xaa can be any naturally occurring amino acid
  misc_feature (6)..(6): Xaa can be any naturally occurring amino acid
  misc_feature (14)..(15): Xaa can be any naturally occurring amino acid
  misc_feature (27)..(27): Xaa can be any naturally occurring amino acid
XDXXGXTPLHLAAXXGHLEIVEVLLKXGADVNA

SEQ ID NO: 11 - protein, 33 aa, Artificial Sequence
  Synthetic Construct
  misc_feature (1)..(1): Xaa can be any naturally occurring amino acid
  misc_feature (5)..(5): Xaa can be any naturally occurring amino acid
  misc_feature (15)..(16): Xaa can be any naturally occurring amino acid
  misc_feature (19)..(19): Xaa can be any naturally occurring amino acid
  misc_feature (27)..(27): Xaa can be any naturally occurring amino acid
XDYFXHTPLHLAARXXHLXIVEVLLKXGADVNA

SEQ ID NO: 12 - protein, 33 aa, Artificial Sequence
  Synthetic Construct
  misc_feature (1)..(1): Xaa can be any naturally occurring amino acid
  misc_feature (4)..(4): Xaa can be any naturally occurring amino acid
  misc_feature (6)..(6): Xaa can be any naturally occurring amino acid
  misc_feature (14)..(14): Xaa can be any naturally occurring amino acid
  misc_feature (27)..(27): Xaa can be any naturally occurring amino acid
XDFXGXTPLHLAAXDGHLEIVEVLLKXGADVNA

SEQ ID NO: 13 - protein, 33 aa, Artificial Sequence
  Synthetic Construct
  misc_feature (1)..(1): Xaa can be any naturally occurring amino acid
  misc_feature (3)..(4): Xaa can be any naturally occurring amino acid
  misc_feature (20)..(20): Xaa can be any naturally occurring amino acid
  misc_feature (27)..(27): Xaa can be any naturally occurring amino acid
XDXXGTTPLHLAAVYGHLEXVEVLLKXGADVNA

SEQ ID NO: 14 - protein, 33 aa, Artificial Sequence
  Synthetic Construct
  misc_feature (1)..(1): Xaa can be any naturally occurring amino acid
  misc_feature (18)..(18): Xaa can be any naturally occurring amino acid
  misc_feature (27)..(29): Xaa can be any naturally occurring amino acid
  misc_feature (31)..(31): Xaa can be any naturally occurring amino acid
XNETGYTPLHLADSSGHXEIVEVLLKXXXDXNA

SEQ ID NO: 15 - protein, 10 aa, Artificial Sequence
  Synthetic Construct
MRGSHHHHHH

SEQ ID NO: 16 - protein, 20 aa, Artificial Sequence
  Synthetic Construct
GGGGSGGGGSGGGGSGGGGS

SEQ ID NO: 17 - protein, 126 aa, Artificial Sequence
  Synthetic Construct
GSDLGKKLLEAARAGQDDEVRILMANGADVNAADYFGHTPLHLAARDGHLKIVEVLLKYGADVNASDFAGKTPLHLAANDGHLEIVEVLLKHGADVNAQDKFGKTAFDISIDNGNEDLAEILQKLN

SEQ ID NO: 18 - protein, 126 aa, Artificial Sequence
  Synthetic Construct
GSDLGKKLLEAARAGQDDEVRILMANGADVNAADYFSHTPLHLAARDGHLKIVEVLLKYGADVNASDFAGKTPLHLAANDGHLEIVEVLLKHGADVNAQDIFGKTAFDISIDNGNEDLAEILQKLN

SEQ ID NO: 19 - protein, 126 aa, Artificial Sequence
  Synthetic Construct
GSDLGKKLLEAARAGQDDEVRILMANGADVNAKDYFSHTPLHLAARNGHLKIVEVLLKAGADVNAKDFAGKTPLHLAANDGHLEIVEVLLKHGADVNAQDIFGKTPADIAADAGHEDIAEVLQKLN

SEQ ID NO: 20 - protein, 126 aa, Artificial Sequence
  Synthetic Construct
GSDLDKKLLEAARAGQDDEVRILMANGADVNAKDYFSHTPLHLAARNGHLKIVEVLLKAGADVNAKDFAGKTPLHLAANDGHLEIVEVLLKHGADVNAQDIFGKTPADIAADAGHEDIAEVLQKLN

SEQ ID NO: 21 - protein, 126 aa, Artificial Sequence
  Synthetic Construct
GSDLDKKLLEAARAGQDDEVRILMANGADVNAKDYFSHTPLHLAARNGHLEIVEVLLKAGADVNAKDFAGKTPLHLAANDGHLEIVEVLLKHGADVNAQDIFGKTPADIAADAGHEDIAEVLQKLN

SEQ ID NO: 22 - protein, 126 aa, Artificial Sequence
  Synthetic Construct
GSDLGKKLLEAARAGQDDEVRILMANGADVNAKDYFSHTPLHLAARNGHLEIVEVLLKAGADVNAKDFAGKTPLHLAANDGHLEIVEVLLKHGADVNAQDIFGKTPADIAADAGHEDIAEVLQKLN

SEQ ID NO: 23 - protein, 126 aa, Artificial Sequence
  Synthetic Construct
GSDLGKKLLEAARAGQDDEVRILLAAGADVNAKDYFSHTPLHLAARNGHLKIVEVLLKAGADVNAKDFAGKTPLHLAANDGHLEIVEVLLKHGADVNAQDIFGKTPADIAADAGHEDIAEVLQKLN

SEQ ID NO: 24 - protein, 126 aa, Artificial Sequence
  Synthetic Construct
GSDLGKKLLEAARAGQDDEVRILMASGADVNAADYFSHTPLHLAARDGHLKIVEVLLKYGADVDASDFAGKTPLHLAANDGHLEIVEVLLKHDADVNAQDKFGKTAFDISIDNGNEDLAEILQKLN

SEQ ID NO: 25 - protein, 126 aa, Artificial Sequence
  Synthetic Construct
GSDLGKELLEAARAGQDDEVRILMANGADVNAADYFGHTPLHLAARNGHLKIVEVLLKYGADVNASDFAGKTPLHLAANDGHLEIVEVLLKHGADVNAQDIFGKTAFEISIDNGNEDLAEILQKLN

SEQ ID NO: 26 - protein, 126 aa, Artificial Sequence
  Synthetic Construct
GSDLGKKLLEAARAGQDDEVRFLMANGADVNAADERGTTPLHLAAVYGHLEIVEVLLKNGADVNAQNETGYTPLHLADSSGHLEIVEVLLKHSADVNAQDKFGKTAFDISIDNGNEDLAEILQKLN

SEQ ID NO: 27 - protein, 126 aa, Artificial Sequence
  Synthetic Construct
GSDLDKKLLEAARAGQDDEVRILMANGADVNAKDERGTTPLHLAAVYGHLEIVEVLLKAGADVNAKNETGYTPLHLADSSGHLEIVEVLLKAGADVNAQDKSGKTPADLAADAGHEDIAEVLQKLN

SEQ ID NO: 28 - protein, 126 aa, Artificial Sequence
  Synthetic Construct
GSDLDKKLLEAARAGQDDEVRILMANGADVNAKDERGTTPLHLAAVYGHLEIVEVLLKAGADVNAKNETGYTPLHLADSSGHLEIVEVLLKHSADVNAQDKSGKTPADLAADAGHEDIAEVLQKLN

SEQ ID NO: 29 - protein, 126 aa, Artificial Sequence
  Synthetic Construct
GSDLDKKLLEAARAGQDDEVRILMANGADVNAKDERGTTPLHLAAVYGHLEIVEVLLKAGADVNAKNETGYTPLHLADSSGHLEIVEVLLKHGADVNAQDKSGKTPADLAADAGHEDIAEVLQKLN

SEQ ID NO: 30 - protein, 126 aa, Artificial Sequence
  Synthetic Construct
GSDLDKKLLEAARAGQDDEVRILMANGADVNAKDERGTTPLHLAAVYGHLEIVEVLLKAGADVNAKNETGYTPLHLADSSGHLEIVEVLLKASADVNAQDKSGKTPADLAADAGHEDIAEVLQKLN

SEQ ID NO: 31 - protein, 157 aa, Artificial Sequence
  Synthetic Construct
GSDLGKKLLEAARAGQDDEVRILMANGADVNAVDIWGNTPLHLAANEGHLEIVEVLLKHGADVNALDHWGDTPLHLAAMWGHLEIVEVLLKHGADVNALDNNGFTPLHLGYGHLEIVEVLLKHGADVNAQDKFGKTAFDISIDNGNEDLAEILQKLN

SEQ ID NO: 32 - protein, 126 aa, Artificial Sequence
  Synthetic Construct
GSDLDKKLLEAARAGQDDEVRILMANGADVNARDSTGWTPLHLAAPWGHPEIVEVLLKNGADVNAADFQGWTPLHLAAAVGHLEIVEVLLKYGADVNAQDKFGKTAFDISIDNGNEDLAEILQKLN

SEQ ID NO: 33 - protein, 271 aa, Artificial Sequence
  Synthetic Construct
GSDLGKKLLEAARAGQDDEVRILLAAGADVNAKDYFSHTPLHLAARNGHLKIVEVLLKAGADVNAKDFAGKTPLHLAANDGHLEIVEVLLKHGADVNAQDIFGKTPADIAADAGHEDIAEVLQKLGGGGSGGGGSGGGGSGGGGSRSDLGKKLLEAARAGQDDEVRILMANGADVNAKDKDGYTPLHLAAREGHLEIVEVLLKAGADVNAKDKDGYTPLHLAAREGHLEIVEVLLKAGADVNAQDKFGKTAFDISIDNGNEDLAEILQKLN

SEQ ID NO: 34 - protein, 271 aa, Artificial Sequence
  Synthetic Construct
GSDLGKKLLEAARAGQDDEVRILMANGADVNAADYFSHTPLHLAARNGHLKIVEVLLKYGADVNASDFAGKTPLHLAANDGHLEIVEVLLKHGADVNAQDIFGKTAFDISIDNGNEDLAEILQKLGGGGSGGGGSGGGGSGGGGSRSDLGKKLLEAARAGQDDEVRILMANGADVNAKDKDGYTPLHLAAREGHLEIVEVLLKAGADVNAKDKDGYTPLHLAAREGHLEIVEVLLKAGADVNAQDKFGKTAFDISIDNGNEDLAEILQKLN

SEQ ID NO: 35 - protein, 271 aa, Artificial Sequence
  Synthetic Construct
GSDLGKKLLEAARAGQDDEVRILMANGADVNAKDKDGYTPLHLAAREGHLEIVEVLLKAGADVNAKDKDGYTPLHLAAREGHLEIVEVLLKAGADVNAQDKFGKTAFDISIDNGNEDLAEILQKLGGGGSGGGGSGGGGSGGGGSRSDLGKKLLEAARAGQDDEVRILLAAGADVNAKDYFSHTPLHLAARNGHLKIVEVLLKAGADVNAKDFAGKTPLHLAANDGHLEIVEVLLKHGADVNAQDIFGKTPADIAADAGHEDIAEVLQKLN

SEQ ID NO: 36 - protein, 302 aa, Artificial Sequence
  Synthetic Construct
GSDLDKKLLEAARAGQDDEVRILMANGADVNARDSTGWTPLHLAAPWGHPEIVEVLLKNGADVNAADFQGWTPLHLAAAVGHLEIVEVLLKYGADVNAQDKFGKTAFDISIDNGNEDLAEILQKLGGGGSGGGGSGGGGSGGGGSRSDLGKKLLEAARAGQDDEVRILMANGADVNAVDIWGNTPLHLAANEGHLEIVEVLLKHGADVNALDHWGDTPLHLAAMWGHLEIVEVLLKHGADVNALDNNGFTPLHLGYGHLEIVEVLLKHGADVNAQDKFGKTAFDISIDNGNEDLAEILQKLN

SEQ ID NO: 37 - protein, 126 aa, Artificial Sequence
  Synthetic Construct
GSDLGKKLLEAARAGQDDEVRILMANGADVNAADYFSHTPLHLAARNGHLKIVEVLLKYGADVNASDFAGKTPLHLAANDGHLEIVEVLLKHGADVNAQDIFGKTAFDISIDNGNEDLAEILQKLN

SEQ ID NO: 38 - protein, 126 aa, Artificial Sequence
  Synthetic Construct
GSDLGKKLLEAARAGQDDEVRILMANGADVNAADYFSHTPLHLAARNGHLKIVEVLLKYGADVNASDFAGKTPLHLAANDGHLEIVEVLLKHGADVNAQDIFGKTPADIAADNGHEDIAEVLQKLN

SEQ ID NO: 39 - protein, 126 aa, Artificial Sequence
  Synthetic Construct
GSDLGKKLLEAARAGQDDEVRILLAAGADVNAADERGTTPLHLAAVYGHLEIVEVLLKNGADVNAQNETGYTPLHLADSSGHLEIVEVLLKHSADVNAQDKFGKTAFDISIDNGNEDLAEILQKLN

SEQ ID NO: 40 - protein, 126 aa, Artificial Sequence
  Synthetic Construct
GSDLGKKLLEAARAGQDDEVRILLAAGADVNAADERGTTPLHLAAVYGHLEIVEVLLKNGADVNAQNETGYTPLHLADSSGHLEIVEVLLKHSADVNAQDKSGKTPADIAADNGHEDIAEVLQKLN

SEQ ID NO: 41 - protein, 103 aa, Artificial Sequence
  Synthetic Construct
MRGSHHHHHHGSDLGKKLLEAARAGQDDEVRILMANGADVNAKDKDGYTPLHLAAREGHLEIVEVLLKAGADVNAQDKFGKTAFDISIDNGNEDLAEILQKLN

SEQ ID NO: 42 - protein, 103 aa, Artificial Sequence
  Synthetic Construct
MRGSHHHHHHGSDLGKKLLEAARAGQDDEVRILMANGADVNAKDKDGYTPLHLAAREGHLEIVEVLLKAGADVNAQDKSGKTPADLAADNGHEDIAEVLQKAA

SEQ ID NO: 43 - protein, 126 aa, Artificial Sequence
  Synthetic Construct
GSDLGKKLLEAARAGQDDEVRILLKAGADVNAKDYFSHTPLHLAARNGHLKIVEVLLKAGADVNAKDFAGKTPLHLAANDGHLEIVEVLLKHGADVNAQDIFGKTPADIAADAGHEDIAEVLQKLN

SEQ ID NO: 44 - protein, 126 aa, Artificial Sequence
  Synthetic Construct
GSDLGKKLLEAARAGQDDEVRELLKAGADVNAKDYFSHTPLHLAARNGHLKIVEVLLKAGADVNAKDFAGKTPLHLAANDGHLEIVEVLLKHGADVNAQDIFGKTPADIAADAGHEDIAEVLQKLN

SEQ ID NO: 45 - protein, 126 aa, Artificial Sequence
  Synthetic Construct
GSDLGKKLLEAARAGQDDEVRILLKAGADVNAKDYFSHTPLHLAARNGHLKIVEVLLKAGADVNAKDFAGKTPLHLAANDGHLEIVEVLLKAGADVNAQDIFGKTPADIAADAGHEDIAEVLQKLN

SEQ ID NO: 46 - protein, 126 aa, Artificial Sequence
  Synthetic Construct
GSDLGKKLLEAARAGQDDEVRELLKAGADVNAKDYFSHTPLHLAARNGHLKIVEVLLKAGADVNAKDFAGKTPLHLAANDGHLEIVEVLLKAGADVNAQDIFGKTPADIAADAGHEDIAEVLQKLN

SEQ ID NO: 47 - protein, 126 aa, Artificial Sequence
  Synthetic Construct
GSDLDKKLLEAARAGQDDEVRILLKAGADVNAKDYFSHTPLHLAARNGHLKIVEVLLKAGADVNAKDFAGKTPLHLAANDGHLEIVEVLLKAGADVNAQDIFGKTPADIAADAGHEDIAEVLQKLN

SEQ ID NO: 48 - protein, 126 aa, Artificial Sequence
  Synthetic Construct
GSDLDKKLLEAARAGQDDEVRELLKAGADVNAKDYFSHTPLHLAARNGHLKIVEVLLKAGADVNAKDFAGKTPLHLAANDGHLEIVEVLLKAGADVNAQDIFGKTPADIAADAGHEDIAEVLQKLN

SEQ ID NO: 49 - protein, 33 aa, Artificial Sequence
  Synthetic Construct
KDYFSHTPLHLAARNGHLKIVEVLLKAGADVNA

SEQ ID NO: 50 - protein, 33 aa, Artificial Sequence
  Synthetic Construct
KDFAGKTPLHLAANDGHLEIVEVLLKAGADVNA

SEQ ID NO: 51 - protein, 33 aa, Artificial Sequence
  Synthetic Construct
KDERGTTPLHLAAVYGHLEIVEVLLKAGADVNA

SEQ ID NO: 52 - protein, 33 aa, Artificial Sequence
  Synthetic Construct
KNETGYTPLHLADSSGHLEIVEVLLKHSADVNA

SEQ ID NO: 53 - protein, 33 aa, Artificial Sequence
  Synthetic Construct
  misc_feature (1)..(1): Xaa can be any naturally occurring amino acid
  misc_feature (3)..(6): Xaa can be any naturally occurring amino acid
  misc_feature (14)..(15): Xaa can be any naturally occurring amino acid
  misc_feature (19)..(19): Xaa can be any naturally occurring amino acid
  misc_feature (27)..(27): Xaa can be any naturally occurring amino acid
XDXXXXTPLHLAAXXGHLXIVEVLLKXGADVNA

SEQ ID NO: 54 - protein, 33 aa, Artificial Sequence
  Synthetic Construct
  misc_feature (1)..(1): Xaa can be any naturally occurring amino acid
  misc_feature (4)..(4): Xaa can be any naturally occurring amino acid
  misc_feature (6)..(6): Xaa can be any naturally occurring amino acid
  misc_feature (14)..(15): Xaa can be any naturally occurring amino acid
  misc_feature (27)..(27): Xaa can be any naturally occurring amino acid
XDFXGXTPLHLAAXXGHLEIVEVLLKXGADVNA